European Patent Application EP 4 169 383 A1, published April 26, 2023. Title: ALTERING MICROBIAL POPULATIONS & MODIFYING MICROBIOTA. Applicant: SNIPR TECHNOLOGIES LIMITED. The sequence listing filed with the application follows.

SEQUENCE LISTING (122 sequences)

SEQ ID NO: 1 - DNA, 5 bp, Bacterial
ttgac

SEQ ID NO: 2 - DNA, 6 bp, Bacterial
tataat

SEQ ID NO: 3 - DNA, 8 bp, Bacterial
tatgaaaa

SEQ ID NO: 4 - DNA, 7 bp, Bacterial
atttgag

SEQ ID NO: 5 - DNA, 8 bp, Bacterial
atttgagg

SEQ ID NO: 6 - DNA, 3 bp, Bacterial
gag

SEQ ID NO: 7 - DNA, 4 bp, Bacterial
gagg

SEQ ID NO: 8 - DNA, 4 bp, Bacterial
tgag

SEQ ID NO: 9 - DNA, 5 bp, Bacterial
tgagg

SEQ ID NO: 10 - DNA, 5 bp, Bacterial
ttgag

SEQ ID NO: 11 - DNA, 5 bp, Bacterial
tgagg

SEQ ID NO: 12 - DNA, 6 bp, Bacterial
tttgag

SEQ ID NO: 13 - DNA, 7 bp, Bacterial
tttgagg

SEQ ID NO: 14 - DNA, 7 bp, Bacterial
atttgag

SEQ ID NO: 15 - DNA, 8 bp, Bacterial
aatttgag

SEQ ID NO: 16 - DNA, 8 bp, Bacterial
catttgag

SEQ ID NO: 17 - DNA, 8 bp, Bacterial
gatttgag

SEQ ID NO: 18 - DNA, 8 bp, Bacterial
tatttgag

SEQ ID NO: 19 - DNA, 9 bp, Bacterial
cgatttgag

SEQ ID NO: 20 - DNA, 10 bp, Bacterial
acgatttgag

SEQ ID NO: 21 - DNA, 9 bp, Bacterial
tcatttgag

SEQ ID NO: 22 - DNA, 10 bp, Bacterial
ttcatttgag

SEQ ID NO: 23 - DNA, 10 bp, Bacterial
atcatttgag

SEQ ID NO: 24 - DNA, 11 bp, Bacterial
tttcatttgag

SEQ ID NO: 25 - DNA, 11 bp, Bacterial
aatcatttgag

SEQ ID NO: 26 - DNA, 12 bp, Bacterial
aattcatttgag

SEQ ID NO: 27 - DNA, 12 bp, Bacterial
aaatcatttgag

SEQ ID NO: 28 - DNA, 13 bp, Bacterial
aaattcatttgag

SEQ ID NO: 29 - DNA, 13 bp, Bacterial
aaaatcatttgag

SEQ ID NO: 30 - DNA, 14 bp, Bacterial
aaaattcatttgag

SEQ ID NO: 31 - DNA, 3 bp, Bacterial
gtt

SEQ ID NO: 32 - DNA, 4 bp, Bacterial
gttt

SEQ ID NO: 33 - DNA, 5 bp, Bacterial
gtttt

SEQ ID NO: 34 - DNA, 6 bp, Bacterial
gttttt

SEQ ID NO: 35 - DNA, 7 bp, Bacterial
gtttttg

SEQ ID NO: 36 - DNA, 8 bp, Bacterial
gtttttgt

SEQ ID NO: 37 - DNA, 9 bp, Bacterial
gtttttgta

SEQ ID NO: 38 - DNA, 10 bp, Bacterial
gtttttgtac

SEQ ID NO: 39 - DNA, 11 bp, Bacterial
gtttttgtact

SEQ ID NO: 40 - DNA, 12 bp, Bacterial
gtttttgtactc

SEQ ID NO: 41 - DNA, 13 bp, Bacterial
gtttttgtactct

SEQ ID NO: 42 - DNA, 14 bp, Bacterial
gtttttgtactctc

SEQ ID NO: 43 - DNA, 15 bp, Bacterial
gtttttgtactctca

SEQ ID NO: 44 - DNA, 16 bp, Bacterial
gtttttgtactctcaa

SEQ ID NO: 45 - DNA, 63 bp, Bacterial
caaggacagttattgattttataatcactatgtgggtataaaaacgtcaaaatttcatttgag

SEQ ID NO: 46 - DNA, 103 bp, Bacterial
aaacaaagaattagctgatctttaataataaggaaatgttacattaaggttggtgggttgtttttatgggaaaaaatgctttaagaacaaatgtatacttaga

SEQ ID NO: 47 - protein, 1053 aa, Bacterial
MKRNYILGLDIGITSVGYGIIDYETRDVIDAGVRLFKEANVENNEGRRSKRGARRLKRRRRHRIQRVKKLLFDYNLLTDHSELSGINPYEARVKGLSQKLSEEEFSAALLHLAKRRGVHNVNEVEEDTGNELSTKEQISRNSKALEEKYVAELQLERLKKDGEVRGSINRFKTSDYVKEAKQLLKVQKAYHQLDQSFIDTYIDLLETRRTYYEGPGEGSPFGWKDIKEWYEMLMGHCTYFPEELRSVKYAYNADLYNALNDLNNLVITRDENEKLEYYEKFQIIENVFKQKKKPTLKQIAKEILVNEEDIKGYRVTSTGKPEFTNLKVYHDIKDITARKEIIENAELLDQIAKILTIYQSSEDIQEELTNLNSELTQEEIEQISNLKGYTGTHNLSLKAINLILDELWHTNDNQIAIFNRLKLVPKKVDLSQQKEIPTTLVDDFILSPVVKRSFIQSIKVINAIIKKYGLPNDIIIELAREKNSKDAQKMINEMQKRNRQTNERIEEIIRTTGKENAKYLIEKIKLHDMQEGKCLYSLEAIPLEDLLNNPFNYEVDHIIPRSVSFDNSFNNKVLVKQEENSKKGNRTPFQYLSSSDSKISYETFKKHILNLAKGKGRISKTKKEYLLEERDINRFSVQKDFINRNLVDTRYATRGLMNLLRSYFRVNNLDVKVKSINGGFTSFLRRKWKFKKERNKGYKHHAEDALIIANADFIFKEWKKLDKAKKVMENQMFEEKQAESMPEIETEQEYKEIFITPHQIKHIKDFKDYKYSHRVDKKPNRELINDTLYSTRKDDKGNTLIVNNLNGLYDKDNDKLKKLINKSPEKLLMYHHDPQTYQKLKLIMEQYGDEKNPLYKYYEETGNYLTKYSKKDNGPVIKKIKYYGNKLNAHLDITDDYPNSRNKVVKLSLKPYRFDVYLDNGVYKFVTVKNLDVIKKENYYEVNSKCYEEAKKLKKISNQAEFIASFYNNDLIKINGELYRVIGVNNDLLNRIEVNMIDITYREYLENMNDKRPPRIIKTIASKTQSIKKYSTDILGNLYEVKSKKHPQIIKKG

SEQ ID NO: 48 - protein, 1368 aa, Bacterial [sequence omitted]

SEQ ID NO: 49 - DNA, 56115 bp, Bacterial
atgaaaatcaccattttagctgtagggaaactaaaagagaaatactggaagcaagccatagcagaatatgaaaaacgtttaggcccatacaccaagatagacatcatagaagttccagacgaaaaagcaccagaaaatatgagtgacaaagaaattgagcaagtaaaagaaaaagaagggcaacgaatactagccaaaattaaaccacaatccacagtcattacattagaaatacaaggaaagatgctatcttccgaaggattggcccaagaattgaatcaacgcatgacccaaggccaaagcgactttgtattcgtcattggcggatcaaacggcctgcacaaggacgtcttacaacgcagtaactactcactatcattcagcaaaatgacattcccacatcaaatgatgcgggttgtgttaattgagcaagtgtatagagcgtttaagattatgcgaggagaagcttatcataaataaaactaaaaattaagttgtgtataatttaaaaagttaatgagatgtggagggattacatatatgaaatattggattataccttgcaatatcatatgatgtttatagagtgtttaataaaggttctgttgcaaagttagaaaaatatagctaattactattttatcatgtcgttgttcccttaactggctaacatatgcctaatttcgtggcatggcgaaaatccgtagatctgaagagacctgcggttctttttatatagagcgtaaatacattcaataccttttaaagtattctttgccgtattgatactttgatatcttgtctttcttactttaatatgacggtgatcttgctcaatgaggttattcagatatttagatgtacaatgacagtcgggattcagtttaaacgctttaattactttagccattgctaccttcgttgaaggtgcctgatctgtaatcaccttttgaggtttaccaaattgtttaatgagacgtttgataaatacatatgctgaatgattatctcgttgcttacgcaaccaaatatctaatgtatgtccctctgcatcaatggcacgatataaatagctccattttccttttattttgatgtacgtctcatcaatacgccatttgtaataagcttttttatgctttttcttccaaatttgatacaaaattggggcatattcttgaacccaacggtagaccgttgaatgatgaacgtttacaccacgttcccttaatatttcagatatatcacgataactcaatgtatatcttagatagtagccaacggctacagtgataacatccttgttaaattgtttatatctgaaatagttcatacagaagactcctttttgttaaaattatactataaattcaactttgcaacagaaccgtattatggaatagagatgttggtaacatttatacaggatcattatacttaagtttaatttcgttattacagaaccacacattccaaccagaagagaaagtatgtctatttagttatggttcaggagcagtaggagaaatctttagtggttcaatcgttaaaggatatgacaaagcattagataaagagaaacacttaaatatgctagaatctagagagcaattatcagtcgaagaatacgaaacattctttaacagatttgataatcaagaatttgatttcgaacgtgaattgacacaagatccatattcaaaagtatacttatacagtatagaagaccatatcagaacatataagatagagaaataaactagtggccgattgtgcttgatgagcttgggacataaatcctaactcgaaataaataagcatatcactaaactgattttttaaagtttacagtgatatgcttatttttttatcttacgattttgtacgtgcatgcttgcctaggggtatggctcgagccctggagccattagtctctcgcacatactattccctcaggcgtcagcacttacaaaatcggttgtaattttcatttttatacgcattcttactgagattatactaataagaggaatagtaaaagcaattctaagtaaaattgcagataagaggtttgttaaaagcagttctaagtaaaattgcagataagaggtacgttaaaagcaattccatgcaaaattgctgataaggggtaagttaaaagcagttctcagtaaaattgcagataagaggtacgttaaaagcagttctaggcaaaattgcagataagaggtgcgttaaaagcagttctcagtaaaattgctgataaggggtaagttaaaagcaatcctaagtaaaattgcagataagaggtaagttaaaagcaatcctaagtaaaattgcagataaggggtacagaaaaactagacttgattacaaaatggagcttgggacataaatgattttttaaaaatgagatgagacgtagattaactccataatcaatacgaatctatcgacttctttatttatgatattcatctctttttaatggaaataaaagtgcgattaatgtgataatacagttacgttaattaaaaaaataaaaatgcaaggagaggtaatatgctaactgtatatggacatagaggattacctagtaaagctccggaaaatacaattgcatcatttaaagctgcttcagaagtagaaggtataaactggttggagttagatgttgcaattacaaaagatgaacaactgattatcattcatgatgattatttagaacggactacaaatatgtccggggaaataactgaattgaattatgatgaaattaaagatgcttctgcaggatcttggtttggtgaaaaattcaaagatgaacatttgccaactttcgatgatgtagtaaaaatagcaaatgaatataatatgaatttaaatgtagaattaaaaggtattactggaccgaatggactagcactttctaaaagtatggttaagcaagtggaagaacaattaacaaacttaaatcagaatcaagaagtgctcatttcaagctttaatgttgtgcttgttaaacttgcagaagaaatcatgccacaatataacagagcagttatattccatacaacttcgtttcgtgaagactggagaacacttttagattactgtaatgctaaaatagtaaacactgaagatgccaaacttactaaagcaaaagtaaaaatggtaaaagaagcgggttatgaattgaacgtatggactgtaaacaaaccagcacgtgcaaaccaacttgctaattggggagttgatggtatctttacagacaatgcagataaaatggtgcatttgtctcaatagaaagttagaggtgagtcttacgtttcagtgacggtagacttacctttaacatgttacatactaaaaaattaatttgaataagaaagagagacatatatgaaatacgatgattttatagtaggagaaacattcaaaacaaaaagccttcatattacagaagaagaaattatccaatttgcaacaacttttgatcctcaatatatgcatatagataaagaaaaagcagaacaaagtagatttaaaggtatcattgcatctggcatgcatacactttcaatatcatttaaattatgggtagaagaaggtaaatacggagaagaagttgtagcaggaacacaaatgaataacgttaaatttattaaacctgtatacccaggtaatacattgtacgttatcgctgaaattacaaataagaaatccataaaaaaagaaaatggactcgttacagtgtcactttcaacatacaatgaaaatgaagaaattgtatttaagggagaagtaacagcacttattaataattcataataaaacagtgaagcaaccatcgttacggattgcttcactgttttgttattcatctatatcgtattttttattaccgttctcatatagctcatcatacactttacctgagattttggcattgtagctagccattcctttatcttgtacatctttaacattaatagccatcatcatgtttggattatctttatcatatgatataaaccacccaatttgtctgcctgtttctccttgtttcattttgagttctgcagtaccggatttgccaattaagtttgcataagatctataaatatcttctttatgtgttttatttacgacttgttgcataccatcagttaatagattgatattttctttggaaataatatttttcttccaaactttgtttttcgtgtcttttaataagtgaggtgcgttaatattgccattattttctaatgcgctatagattgaaaggatctgtactgggttaatcagtatttcaccttgtccgtaacctgaatcagctaataatatttcattatctaaatttttgtttgaaatttgagcattataaaatggataatcacttggtatatcttcaccaacacctagttttttcatgcctttttcaaatttcttactgcctaattcgagtgctactctagcaaagaaaatgttatctgatgattctattgcttgttttaagtcgatattaccatttaccacttcatatcttgtaacgttgtaaccaccccaagatttatctttttgccaacctttaccatcgattttataacttgttttatcgtctaatgttttgttatttaacccaatcattgctgttaatattttttgagttgaacctggtgaagttgtaatctggaacttgttgagcagaggttcttttttatcttcggttaatttattatattcttcgttactcatgccatacataaatggatagacgtcatatgaaggtgtgcttacaagtgctaataattcacctgtttgagggtggatagcagtacctgagccataatcatttttcatgttgttataaatactcttttgaactttagcatcaatagttagttgaatatctttgccatcttttttctttttctctattaatgtatgtgcgattgtattgctattatcgtcaacgattgtgacacgatagccatcttcatgttggagctttttatcgtaaagtttttcgagtccctttttaccaataactgcatcatctttatagcctttatattctttttgttttaattcttcagagttaatgggaccaacataacctaatagatgtgaagtcgctttttctagaggatagttacgactttctgtttcattagttgtaagatgaaatttttttgcgaaatcacttaaatattcatccatttttttaacggttttaagtggaacgaaggtatcatcttgtacccaattttgatccatttgttgtttgatatagtcttcagaaatacttagttctttagcgattgctttataatcttttttagatacattctttggaacgatgcctatctcatatgctgttcctgtattggccaattccacattgtttcggtctaaaattttaccacgttctgattttaaattttcaatatgtatgctttggtctttctgcattcctggaataatgacgctatgatcccaatctaacttccacataccatcttctttaacaaaattaaattgaacgttgcgatcaatgttaccgtagtttgttttaattttatattgagcatctactcgttttttatttttagatactttttttattttacgatcctgaatgtttatatctttaacgcctaaactattatatatttttatcggacgttcagtcatttctacttcaccattatcgcttttagaaatataactgctatctttataaacttgtttgaaatttttatcttcaattgcatcaatagtattattaatttctttatcttttgaagcataaaaatatataccaaacccgacaactacaactattaaaataagtggaacaatttttatctttttcatcaatatcctccttatataagactacatttgtagtatattacaaatgtagtatttatgtcaaaataatgttataatttttgtgatatggaggtgtagaaggtgttatcatcttttttggttctgttgcaaagtaaggttctgttgcaaagtaaaaaatatagctaaccactaatttatcatgtcagtgttcgcttaacttgctagcatgatgctaatttcgtggcatggcgaaaatccgtagatctgaagagacctgcggttctttttatatagagcgtaaatacattcaataccttttaaagtattctttgctgtattgatactttgataccttgtctttcttactttaatatgacggtgatcttgctcaatgaggttattcagatatttcgatgtacaatggcagtcaggtttaagtttaaaagctttaattactttagccattgctaccttcgttgaaggtgcctgatctgtaattaccttttgaggtttaccaaattgtttaatgagacgtttgataaacgcatatgctgaatgattatctcgttgcttacgcaaccaaatatctaatgtatgtccctctgcatcaatggcacgatataaatagctccattttccttttattttgatgtacgtctcatcaatacgccatttgtaataagcttttttatgctttttcttccaaatttgatataaaattggggcatattcttgaacccaacggtagaccgttgaatgatgaacgtttacaccaagttcccttaatatttcagatatatcacgataactcaatgcatatcttagatagtagccaacggctacagtgataacatccttgttaaattgtttatatctgaaatagttcatacagaagactccttttggttaagattatactataaattcaactttgcaacagaacctcttaatcttattggatacaataactaacttaaacacattatctacaagtaaaaacttgtaaaaagaacatgtgttcttaattagtgtataattagtttaaattgattatggggtgatgtaatgaatgagagtaatcaaattatattcgatcatataacaaaggctattgaaaatatgaaaaataaaggctgggaaacaaggtatgggcaagaaactttaatgtatgatgtatttgatgcttatgattcaagagaaaatttaatagtagaagcgcaagtaggtataggaaaatcatttggatatttaattcctggtatattgatttcaaaaagtactaaaaaacctttaattgtaacgacttcctcaattcaattaactgagcaactagtcaatgatatacagcaagttgaagaaattttacatatatctgttgattgtatagtaggtaaaggtgtaactaactatccttgttttaaagaaattcatcgtaaaaatttaagtaaattaaatttaatggaggctttagatatagcaaataatggtttaacaaaacaaactgtacgtgagactaatttaaaatggaatcaaatatctaccaataattgtattatgagtaaatgtcactataaaaatgaatgcgcttattttaaaatgagaaataagttaaaagagggaaatagatatattagactcaatgaatataagccgaaagtcataatcgttaatcaagatatgttaatgatgaattttaaaaagttaacctttggaaaagagagtttaatctatgatgatccttgtatgctaatcgtagatgaagttcacaacttagaagagaaacaacgtgctaacatgactaaaactattaactctaaaactatgataaataaaataaaagaaggcgcaaaccgagttggtagtagatctcggtatttaaaaaatataaaaatgattgaagattggtttaatcttcaaaaggatagtgccaaaagtgagatatacaaaaatggtaattgtttatctactggacgagttgatataaaacctgttagtcatcatcaaatggccaaattaattagtatgacaaaggaaatagttgaagaattcgatgttaataatattgttgtatttaaacaatcttcgttagttagtaatgaacaattagaaatagctaataatctgttaacattatttaaaaatcttcaaaataacagcgacaaatatatattttggactgaaataactaagcaagaccaaattgatatttcattttgtcccaataatattgctgaaacacttagaaaaacagtttttagtacaagttacccagttgtatgtctttctgcaacaattactaataaaactaataatgaaaatagctatgagtacattaaagaaataattggttttaaaggctatgaggaagatattaagtataatgattttccgtacaaggaaagcaggctctacatacctccaaacttaccaaaatttgataaacgtgatgttaaatattatgaagaaataggtaaacatatttttgaattggcaagccaaaataagggaggcactttgatattgtttactgctaaagatgacattgacggtgtatataatgatttatcaaaaaggaaatttaataaaactatctatgtagatgatggtagtaaaagtcaaaatgaaattattgaatcatttaaaaaaactaaaggtgtaatattgggtacgggagtattttgggaaggaatagacttaaaaaatgaattattaacattattagttattgtcagattaccttttcctacgattgatccaattacaaaatataagattactaaattaaatgatagtaatgaagcagttatagttcctgaaatgataattaaactgaaacaaggtgtaggaagattagtaagaacaaagcaggataaaggtttattagtgttattagattcaagaatgaataaacccatttataagcataaagaagcagtattagatgcattaccaattaaaaatatgattcataaagatgaagtcaaagatttccttaataacatttaaagtaagtagtaatagttatccaatattttctagttgattctcttataatatgtccaattaagtgtagacgattcaagatgatattgagggaaggatgagaatgtgtcttttaggtagctcatttgatgataaccttaaacataatatttactttcatcctgctgaaaaaagaggttacagtttcaagccgatagaatacattgggctatataaagacaaagcaataaaagctatcggaaaagtagacaaagtaatagtgacggaaataaatgagagctcattatccttgaagacagtttatcctgtaggtactgagttatcgattgatgagtatgaaatagttaaaaataaaataatggtgcttgggaaagaaaagtggactaatctattgaacgaaccccattattattacttaattgaagattttatagagacagactacaagaaaacatctaaaggtggatcgatgggagttaagtattttaatgtgaatgaaattttgaatagggattgcttaaccaccgaacaaatcgctaaagaattatgtaataaagattgggaatgataaatagtgaatgaagctataatgcaataatgtatgtataacataatcaagtaatgaaattaatgataagggagtatggagtaaagaattgaattagtttgcatggtctatgtatcttaaaggtgttgaaggagatacaccgaagtatgcagtaccaattcttgaaacagactttagtgatttaccatctacacatacgacagtcggatcacttgatcggtttcgagataagacaatgagcattaacagaagcgggagtaactgttgaattccatttatatccagttagatactagagtttgaagtgataaatcttgattcggatgctgaaataagtaaaagagcagttactgaatataatataagtataagtatgccactagatattttaaggggtatttattcacttttataaaatcatctgctaagatagtgtggaagatttttataggagctgattataatgcgacatataaatatgtcatacatcatacgctatagtactctaactcaaagataagaagtacttagttatgaatagcattcatttcacaaagtacttcaacaaaaatggaggaatatgaaatgaataaaatagaagtgtataagtttgttaaagtaaagcagttagtatatcaattgattaagttatatcgtacaaacgatatgaattcccataaaacacaaaaagattttttactaaatgaaattaatgatatctttaaagaaaaagatattgatatctcggactttattacatcgattgacgatgtaaaattaactaagaaaaaagcagaacatcttttaaatgaattaaaagtgtacatccaagattttgaaataccttcatcaagtcaactggagaaaatttttcgtaaagtaaaaaaattaaagagaccagatataaatttaattgatacaaaagaaatttcatatttaggatggaatgataattcttctaaccgaaaatatatcgtttataaaaatttagatgataaattcgaaggtatatatggcgaaatttcaccaaataaagtaaaaggattctgtaaaatttgtaatcaggaatctgatacatcactctttctcaataaaactaaacataataagagtagtggaacatatactaaaaaaggagattacatttgttatgacagttttaaatgtaatcagaacctagatgatataaataatctttacgaatttattgttaaaataaaatagatccaaacagccctgatctttagaactaatgatcagggttgttatattttgtacctcactcttaatcgatacgctgagccttataataaataaagctaagattggttagtgtgtaactttatgcaatttgaaaagatataatgaaataagagagttttggtgatgatattaatatttaaatagatctatagacaattaatcgctgttgatttttaacaaatcaattcaatttagttatgttttgtgatggcatactaattaaaaaaagaagaactaggttttgtgccctagttcttctttttatttaattgttattcctatttcttaataagcgtaatgaattaagtatgacaagtatcgcagcgcctgtatcacttaatactgccaaccaaagtgttaatagcccaggaaatacaagaatgaatgcaatcaattttatgatgatagaaaaatatatgttttgcttaatgatatttttagcttttttacttatagaaatcgtacgtgttaattgatttatatcatctgacataagtacgacatcagctgtttccattgctgtatctgaaccaatacctcccattgcaatacctacgtcactttgtgctaaagcaggggcatcatttatgccgtctccaatcatagcgacacgatatcctttattttgcaaatcttttattgcagctaatttgtcaccaggcattaattcagcataaacttctttaatacctgaaagttgtgcgattttttgggcagtacctttattatctcctgttagcattatagtgtttttaatgtgagtaccatttaattgttgtattatttgcttgatatttgaacgtaatgggtctgcaatagtaatcaagccatgaatcatgctagaagatgcaataatgatgacggtaaaaccttcttgctcatatttgtttatttcttctttatagttgttaatttttttgttaatagactcaattaattttacgttaccagcataaacgtaactttcatttattttacctttgatgccttgaccaacgatattttcaaaatcagttacataagcttttttaacatttaattgcattgcgtaatctacgatagcgttgctaatagggtgggttgagtaggattccaaactcatagcaatatttagcaatgttgtttcattagcatctatagttttaatcgtatccacctttggacgaccttcagtcaaagtacctgttttatcaaaagccaacgcagataaagtacctagaccttctaaatggttaccacccttgataagtacgccattttttgctgcacttccaatcgcagtaacgatagctaccggtgttgaaatgacaagtgcacatggacatgcgataactagtaattcaagccctttatataaccattcgccccacgtacctaaagagaatagaggtggtatgaccatgactaataatgctaatacaaagacgataggtgtataaatttctgaaaatcgatctataaaagcttgcgtcggtgctttattttcttgtgcttcttcaaccatatgaatgattttagaaagcgttgtatcttctaccaatttagacacccggatgtataaagtaccattttcattgatagagcctgcatatacttcatcgttaatcgttttatcaacaggtatcgattcaccggtaataggtgcttggtttaaactggaacttccatcggtaattgttccatctaaagggacgcgatcacctggtttgataagtaagatttcaccaactcgtatatctgtcaaatctttagtagttgttccgttttctgttatgacatttgctgttgtggaagtaatatccattaatgattgtatagaattacgtgttttatctattgaaattgtttgcagcaaggttccaattgtaaataacaatacaacaatcgcaccttcaaaatattcaccaatgaatatagcgccaataacagctacggacatcaacacattcatatctaagcttttagatttaatggcataatatgcgcttttcaatggttttatgccactaacaataatggctatgatatacattaaatttgcaattaatactggcaatgttgtcagagttacaactaaaccaaggataagaaataatgttgaaatgataggttttctgaatactctccatttggaattactacttttttttgttggacttaatgttgcagaataaccgattttagaaacttctttttcaatatttttagttttattaccttcaaaaggttctgttgcaaagttgaatttatagtataattttaacaaaaaggagtcttctgtatgaactatttcagatataaacaatttaacaaggatgttatcactgtagccgttggctactatctaagatatacattgagttatcgtgatatatctgaaatattaagggaacgtggtgtaaacgttcatcattcaacggtctaccgttgggttcaagaatatgccccaattttgtatcaaatttggaagaaaaagcataaaaaagcttattacaaatggcgtattgatgagacgtacatcaaaataaaaggaaaatggagctatttatatcgtgccattgatgcagagggacatacattagatatttggttgcgtaagcaacgagataatcattcagcatatgcgtttatcaaacgtctcattaaacaatttggtaaacctcaaaaggtaattacagatcaggcaccttcaacgaaggtagcaatggctaaagtaattaaagcttttaaacttaaacctgactgtcattgtacatcgaaatatctgaataacctcattgagcaagatcaccgtcatattaaagtaagaaagacaaggtatcaaagtatcaatacagcaaagaatactttaaaaggtattgaatgtatttacgctctatataaaaagaaccgcaggtctcttcagatctacggattttcgccatgccacgaaattagcatcatgctagcaagttaagcgaacactgacatgataaattagtggttagctatatttttttactttgcaacagaaccctttttgcaataatacatttaattaaaaccttgttttaaacatcgatgacaagatctaatgtaggacgtggagacatcattttcggaatgatataaataaatccataaatggagataaatcgaaaacatttatacccatagggggtatgtgttatagtataagtatagctaatataatattttcataaataggaggggttaatttgaataataatggtgaagagcataatcctcaaaatcacatgaatcattccaatcacatgcatcatgataaccatgcctcacatcatcatagtggccatgcacatcatcatggaaattttaaagttaagttttttgtttcattaattttggcaatacctatcattcttttatcgccaatgatgggtgttaacttaccttttcaattcacatttccaggttctgaatgggtagtgttaatattaagtacaattttattcttttatggtggtaaaccgttcttgtctggtggtaaagatgaaattgctacaaaaaaaccaggcatgatgaccttagttgccctaggtatttcagtagcttatatttatagcttgtatgctttttatatgaataactttagtagtgcaactggtcatacaatggactttttttgggaattagcaaccttaattttaattatgctattaggacattggatagaaatgaatgctgtcggaaatgctggagatgctttaaagaaaatggcagaactgttacctaatagtgctattaaagttatggataatggccaacgcgaagaagttaaaatatcagacatcatgactgatgatatcgtcgaagtaaaagccggagaaagcattccgacagatggtattatcgttcaaggacaaacatctatagatgaatccctagtcactggagaatctaaaaaagtacaaaaaaatcaaaatgacaacgtcatcgggggttctattaatgggtctggaacaatacaagtcaaggttacagctgtgggagaagatggatatctttctcaagttatgggacttgttaatcaagcacaaaatgataaatctagtgctgaattgttatctgataaagtagcgggttatttattctactttgctgtaattgttggcgtgatttcttttattgtctggatgctcattcaaaatgatgttgattttgcattagaacgtcttgtaactgtgttagtcattgcttgtccacatgctttaggcttggcaatacctttagtcactgcacgttctacttcaattggtgcacataatggtttaattattaaaaatagagagtctgtagaaatagctcaacatatcgattatgtaatgatggataaaactggtactttaactgagggtaacttttctgtgaatcattatgagagctttaaaaatgatttgagtaatgatacaatattaagccttttcgcctcattagaaagtcaatctaatcacccattagctataagtattgttgattttgcgaaaagtaaaaatgtttcatttactaatccacaagacgttaataatattccaggtgtcggattagaaggtctaattgataataaaacatataaaataacaaatgtctcttatcttgataaacataaacttaattatgacgatgacttatttactaaattagctcaacaaggtaattcaatcagctatttaattgaggatcaacaagtcattggcatgattgctcaaggagatcaaattaaagaaagctcaaaacaaatggtagctgatttactatcaagaaatattacaccagtcatgcttacaggtgacaataatgaagtggcacacgctgtcgcaaaagaattaggtattagtgatgtccacgcacaactcatgccagaagataaggaaagcattataaaagattatcaaagtgacggtaataaagtcatgatggtcggagacggtatcaacgatgcgccgagtcttataagagccgatattggtatagcaattggtgcaggcacagatgttgcagtagattcaggtgatatcatacttgttaaaagtaatccatcagatattattcatttcttgaccctttcaaataatactatgagaaaaatggtgcaaaacttatggtggggtgcaggttataatattgttgctgtacctttagcagctggtattttagcgtttatcggcttgattttatcacctgcaataggtgctattttaatgtcgctaagtacggttattgttgcaattaatgcctttacattaaaattaaaataaaagataggagttttattatgattaaaaaattattttttatgatattaggatcattactaatattatcagcttgctccaataatgatgaaaaagataaagacactaatgaccaaaaaagtgagagccatatgaagcataatgatgaaagtaaagttcctgaaggtatgaaatcgactaatgagggtgaatttaaagtaggagataaagtaacgattacagcagggcatatgccaggtatgaaaggtgcagaagctactgtaaaaggtgcgtataaaacatatgcttatgttgtaagttataaacccacaaatggaaatgaaaaagtaaacaatcataaatgggtcgtaaacgaagagatcaaagatgcacctaaagatggatttagtaagggcgatactgttaaattagaagcaagtcatatgtctggtatgaaaggtgctacagtcaatatagataacgtgaaaaagactactgtttacgtagttgattacaaatccaaagataatggtaaaatcattaaaaatcataaatggatgacaggaaatgaactgaaagcacgataaaaatctagttctagattgagaaataaatagatataaagatatcctccttaatcaataatttaaataacttattattgttaaggaggatattttttagtgtgtaaattaaaaagaattttagaagaataacatttatcaaaaaactgttcattaccttattaaatgaaattatataattaaaaaccgcatcattaaccgatacgcagaagcgtaccacaaataaaactaaaaaatagattgtgaaaaatttatctttgaaaggggtcgaatgagagacatagaagtagaaaaagcctataagatgatgaaagaacaaggtaaaataaattttagtgaataccataagacactattacatatacatactctaggatcacatgatttaaaattatatgatgaatggaacaaacaatatttctatctattagccaagatgaaatatttagaattgctaaaaaagaaaatattctttacagtgagtattctaatataaatgatttaaaggaattagatatttttaagaactataaaaatctaaaggaaatgctttcttattttattttggtatacagcatatatactaatggaatatcaatagttgttgttgcagatcataatactgtgtgaagaatggaataaagaattctgtacggcttctgttctactcttttttattaaaaatatataataaagaattttttaaaatagtaaaatttatactttgattaacttttgacataattatgaacatctaaataagtaaaaatcaaatatttgaaattgtgttaatatgaatgtagaaactaaggtaataatttcatttaaaatagcttttaaaatttatatacatattagcgttgtgatacacgtagaaagggggaatcaaaagtggaaacgctaatggttaaagcaatggggacggtgatacgtttatcgattgaacatcaacattcgagtacattacttcaagaagctgaattaaaaattcatgattgggaatctcaatttagtgctaatgatccaaaatcagatttgatgaatgtgaatcaacatgcaggtatcgcaccagtcaaggttaatcctgagatgtttaacatgatacgttatggttatgaaactacactatcttctaattttaagatgaacatattgatagggccattagttaaattatggaaaattggtttcaaagatgcattgaaacctaaagaagaagatatacaacgcgctttaatgtgtatgaatcctgaaaatcttgttctaaattcaaagacacatgaagtatttcttacacgaccaggaatggagattgatttaggagccattgtaaaaggttattttgctgatcaattacagcaatactttttatctcatggtgtagcttctgccattatcgatttaggtggtaatgttttaacaattggtagacaaccggaaactctagaaaaatggcatgtaggtatacgcaatcctttttataaagatgcattatcactcgttacattaaatgtagagcatcaatcagttgttacttcaggcatctatgaacgctatttcatacaggaacatcaattatttcatcatattttggattccaatacagggtatcctgtagataatgatatcgctagcgtgacaatcatatctgatcatgggattgatggcgaggtatggagtacaatttgtagttttggtcaatcacaacaaaatattgaattattaaacctcatagatggtgttgaaggcatcattgtgacaagagatggaaacgttttaatgacttcaaaaatgcaaaggtatttataaaattttaaaaaatactcataaagagtattttatttttaagtataaatgtgaaaaaaatcacaatgtattaggaggaattgctatgagtaaagaattatttgatacttttaaatttaaatgtggtgccgaattaaaaaatagagtattaatggcgcccatgactatccaagctggatattttgatggaagtgttacatcagaaatgattgattattatcaatttagggctggtgatgcttcagcaattattgttgaaagttgttttgttgaaaaccatgggagaggcttcccaggagctataggtattgataacgatgacaaaatacctggacttaaacgtctagcagaagcgattcaatctaaggggtcaaaagcgattttacaactttatcatgctggaagaatggcgaatcctaagttcaatgaaggtgaacaacccatatctgcgagtcctattgcagcattaagacctgatgcggtaccaccaagagaaatgacacatgctcaaatcaatcagatgatagaagatttcggagaagcgacacgtcgtgctatagaagcaggatttgatggtgttgaaattcatggtgccaacacatacttattacaacaatttttctctccgcattctaatcgaagagaagatacatggggaggcagtcgtgaaaaacgtacgcgattcccaatcgaagtactaacaaaagttcaacatgtcgttgatgaaaatgaagcttctcaatttataataggatatcgattctcacctgaagaaattgaagagccaggcatacgttttgaagatacaatgtttttactaaatactttagcaaaatatgaacccgattacttccatatatcagcaaacagttatcaacgtacgtccatagtgaatcaagaagatacagaacctttaattaataaatatcataaaatgcaaagtgcacaattggcacaaattccattaatcggtgttggtagtattgcgcaacgaaaagatgcagaacatgcccttgaactcggttataatcttttaagtgttgggaaagcctatttagtagaacctcaatggacggataaaatttcacaaaacgaagaagttgaacaatttgtcgatatacatgaccaaaaaatacttcacataccatctcctctatggaaagtgatggacttcatgattttagataaagaagaagaacatcgtaaatatgaaagattaaaagcactacaaaataaaaaagtgaaatttaacaaaggcacgtatcatgtttatgcaaaaggtcataatggcaatctaccaatgaaagttcaattgtcggaagataaaattgtaagtattgaagtagatgatagtggagagtctgaaggtatagcgaacccagtttttgaacgtttacctcaagatatcatcaatggacaaacgttaaatgtcgatgtcatatcaggtgcgacagtaacaagtgaaggcatcgtacagggcattgcagatgcaattgaacaagcaggcgaagatccagatattttacgagcacgtcctaaaccagtcgttcagtggtctgatgaggtcgttgaagagacgactgacgtagtcgtgattggtacaggtggtgctggtttaagtgcagctgctacggttttagacgaaggaaaagaagtcatcatgcttgagaaatttgcggctataggtggcaataccatccgaacaggtggtcaagtcaatgctgctgagcctaaatggcaaagtgcattccctgcactcgctggtgaaaaagacacattgatacagttattaaatcatgatgaaaaggatatagatgaggcttatcttgaagatttcaatactttaaagcgtcaaattaaagattaccttgaaaaaagtagcaataaagatgattatcttttcgattctgttgaattacatcgcattcaaacgtatctaggtggaagacgtaaagatcgtaataatgtcgaaatttcaggtgattatgatttagttaaaacactcacagataatgttttggaatcagtatactggttgaaagataaaggggtacattttgatcgttcatttgtagatatgcctgttggtgcactatggcgtcgtggtcataaaccaatgaaagcacaaggtttagagtacattgaaaatctaggagactacgttaaacagcatcatggtcgtatttttacagaaactactgcagaaaaattaattaaagaaggtaatcaagttgttggtattgaagcacgtaaagcaaatggtgctaaagttaagattcacactcgtcacggcgtagtgttggccacaggtggttttggagcgaatactaaaatgatacaacaatataatacgtattgggataacattccagatgatattaaaacaacaaattctcctgcaattacaggtgatggtatacgtttaggtgtgcaagcaggcgctgacatcgtaggtatgggattctctcaaatgatgccgatttctgatcctaagacaggtgcattattcacaggattaatcgtgacaccttcaaacttcgtcttcattaataaggaaggccatcgttttgttaacgaatttgaaagtagagatgtattatctaaggcagcattagaacaaaaagacggcatcttctatattattgcagacgcaaatattaaagcgctagctatgaatacgactgaagacaaaataaatcaagaattagaagatggcactttaataaaagctgataccttagaagtgttagctcaaaaattaaacatagatgcaactacttttgtgaatacgattgaaagatataatactttcgtagaactaggacatgatgaagatttcaataaaaatgcatttgatttaaaaatcgaaaaagcaccattctatgcgacaccacgaaaacctgcaatacatcatactatgggtggtttgaaaatcaacatacatgcacaagtcgttgatgtagaaggtcatatcattaaaggattgtatgcagctggtgaagttgctggtggtatacatgcgggtaaccgtctaggtggtaatgcactggcagatattttcacttttggtcgcatcgctggtcaaagtgctgtaatgaaataaataaagaagaacaggaggacatttaatgatgagtgaacagtttaataaaggaaaacaactcattgtagcgattattttagggattctcacatattggttgtttgcacagtctttcttgaatatcgcaccacatgttcaacgtttctatgatgtagatatgagtattgttaacattgcggtcagtctcacatcactcttaactggtgtatttatagttgtagcaggaggtttatctgataagttaggtcgagttaaaattacttacgcaggtttgatacttagtatacttgggtctattgcactgattatatctcatgcgccacttttattattggtaggtcgagtgttacaaggtttatctgcagcatgcctacttccagcaactattgcgttaattaattcattctttcatggtgaagaaagacaaaaggcactaagttattggtcatttggttcatatggtggaacaggattagcatcactatttgctggaatgatagccacttttattgagtggcgttggattttcgtgttgtcaatcattttctcaattcttgccttaatattgcttaaaggcataccagaatctaaagatgaatctgcacataataaaaaatttgatattattggtattattatttttgtcattatgatgttaagtattaacatagtaataacccaaggtgatagaattggatggttaaatcctattattgtaatattaattgccatattcattgtgacattaatagctttctatatatttgaaaaacgtcaaaatgaacctttcatagattttagtttattttcaaataatatttatattggcacaacattagctaatttaatggtgaatatggatataggctcacttgcattatttaatatctatgttcaagatgataaacatttaacaggagcacaagcaggtttaattacaattccatatatgttgtgtagtttattaatgatacgtgtaggtgaacgttttatgcaaaatcgaggaccgcaattgccacttatgctaggtcctatatcaattacagtgggtattatacttttagccttcacttcgttgcctaacatgatttattatattgtagcgtgcatcggctttatctttataggtttaggattaggtttctttgcgacaccagcgctatctacagctgtatctaatgttccgtcagaaaaagcaggtactgcatcagggattatcaaaatgacttctacactcggtgcagcatttggtatcgctgttgtaactacaatctatacggcattgtccgtcaatcatccagcacaatttgcagctacaatcgcatttatcgtgggggcaggtttagtgtttatcgcatttattgccgcgtattgtttaattcctagaaagaatgtagatgcttaaatcgagagttggcgcagtaaatatcattgcttgaattttgatcgtatgttgaatgatgaataaatagttaaacttgatgatagtcttgaaataggagatgcgtttgaagccttttcttcagaattacgcttggaagatatcaatcaccatccgctgttgcaaacttagtatcattcttagcttctaatgattctgactatattactggtcaattcattttaactgatggtggattagtgtatagataaaaagggatacttcgtcatgataattaatggataaaaaaagcgtttaaatatttatatataatgattgtgtgcttatacaaaatgtcaactcaatgcattcatgtgagagtgggatgatgagtctgagacataaagtctctggataagtcaataaagacaatttctattgaaataatatagaaattgtcttttttataattttttgattattttcagattattgagctgctacttttcttatattgagtgccattaatacaaatccaagttctcttttaattttatttattcctctaatggatattcgaatgaaacccgttctagtaatttagttttgaacccacctaaatgaatatatgagttattttttatactataaaatatattcagatttcaatagtgacataaaataggcatctttatatttacctttagtgtagaattgctctttgagtaatccttcagttttaaatccttgtgattcgtatatatgcacagcttttttgttatctgtatcaacatatagataaattttgtgcatatttaatatatctaatgcataatttatcgctttttcgaatgcgaattttgcataacctttaccactgaactcaggtttaataattatttgtatttcacaattacgatggatgtaattaatttctactaattcaacaattcctatgacttgattttcatcttcaacaataaaacgtctctctgattcatctaataaatgcttatcaaataaatattgaagttccgttaaggattcataaggctcttcaaaccaataagacataatagaatattcattatttaattcatgaacaaaaagtaaatcactatactctaatgctcttagtttcataattccactcctaaaattttcctatatatttgcattataaatataaataacgaataagttatcattcactgtgaatactctattttaacaattcactacatactaattctcattttcttattattctctaatatctctgatttattactcttactatgaaacatataaaactgtcacatttgtttatattaataataaatacatcaatgataacaaaaagaaaataaaaaaataaaaatagagcatccctcaccgtaaaagtgaaggatgctttatttttattagaatatagttttcattttgatagataatggttaataattgtctataaatcattattaaggaccgttgtaatacaatcgtcattcataaaattttcatagattttatccaatattttttcatcttcaattgctgtgaaatgatatactagcccttttactattgatacatactttcttcttatgaggttttagcatttccatcacttgttcgacacgttctacaacaactggtcgcttcgcataagcaccataagctagaatcactgtgtcactttcgctaatcgctttcatcaagtgaatatcagtgtgctcatcgtatggatttttgatgtgtttgagattttctggacttttaatattagagaatagatttacaagatatacagcaccgtatctttctgaattagctaattggttgaggatgagaacagttgtgagatcgagtgataatacaccatctaaatgaggatacatcgttatcactgtacaaacaggtttcttttcatcccacgtctttttgagtaagtatcggtgtttttcatcgtcgctaaatatcgcttctgtgtatatcgtacttttgattgtattcatcatcttcactccttttagtattcttctggtaaaagcatcacataataaaaagtgtctacatcatcttcacgaatgacgtagactttcttaggtactgcattttgattttttacatagtttgtatagtgatattccaatttgtatgcgggctgttcttgttcatgagtaatagagagtatattattatcttcttgtagtttaaaaatgtgtaggtaatctgtatgaccttgttgatctctttcttttaccatattccaaagtaagatttgaaggtctagagatagttgttcactaatgcctcttgtgatgtatcgattgattttcatactattttcctccattttgcttttctttcatgatgtcaatcacttcgttaatgactgtaacagatatttatgccactttgatccaattattcatagttattccctccttctcttagtaaatgacgttcatcgataatcgtatttttagtatctgtgaggtatagaaagtccatatcaaaatgatccagataaccaatgctgatgagttggttattggcgtacattagaaatggatagatacttagctcatgtagctcattattatagtaggtataagtttcaagtatgagatgtgccagtggagaattattaataaaacgttccggtagaatattttctgctgcttcttctaacgcttcacattcccatgtttcgttgttagatagttggaatagatgagttatatattgtttgagttcttgagtgattgtttccatatcattgcctcctagatagtgtgatagtgatgtagttcatatacatcaatgggataatatatatttgatttgtcatttattacgaatcccggtaagaataagagaaaattccgatcaaaaacccgtgataaacgttggtgtaacaaggaaatcccggaatcccactcattttgacgaacaatcaactcattatttataagtattgatgatagggttgggtttctgcttccttatatatattatttatttataaagaataacgggattttgggattgtgcttgcacaatccttctgcttcttcgagtaagcaaatcccattcatttcccgttaaaaaatcatcgtgggatgttctttagcaatttcaatataagcttcgtgtagtagtagatagataatgcaatttgctaccatattagataagtgttattgaaattgataaagagaattcttataaatagttataaaaagtaatcagaagaagaaaataaagaactttctataataaaaagtcttcactattaaattttagtgaagactttttacttaaaattttattatttataaaactaagccaataatacttgctgaaataattgatgctaatgttgcacctaataataatcttagggcaaaagaagctactttatttccctgtttactatcaatacctttaatagctcctaccataattccaacagtaccaaagttagcaaagcttacaagataaacagatattataccttgagtctttggagatagagaagaggcaattttttgaaaatctaacattgctacgaactcatttgtaattaactttgttgccataattgatccagcacgtatagcttcactccatggaatacccataatgaaagcgataggagcaaatatgtaaccaatcaattttttaaaatctagaccgactaaatcaaatacaatagtaattcctttcattaaagatataaaagctaacaacattattgctacagtaatagcaattctgaagccatcaatagcactttcaccaatcatttgaaagaaagttgtttttttaatatttttttctgattcagcttctaattctttattatcatttttgtaaggattaatgacgctagcaattatcaaagcactgaaaatatttaaaacaactgcagtaactacatatttaggatcgatcatttgcatatatgagcctagcatagccatactgacagcactcatacctgaagtagcgatagtatataacttttcttttgacaagcttggaataatatttttaactgttaaataaacctctggttgacctaacatagaagtagatattgcgatatagctttcaagttggcccatatgagttattttattaattatccaacctataattttaattagaaaaggtaaaattttaaaatagtttaacataccaattaaaactgaaataaaaactaaaggtagtaatacatttagaaagaaattatagccgtttttattttgtaaatctccaaaaacgaattcaataccttctttactaatattcattaaaccttcaaaaaatgtactcattgcggttaataaattaagacctattgatgtattcatcataaataaaacaagaacaatttgtattactatcataatcattggtttttttatatctatagcttttctattaaaactaaaaatatatgcaactaataaagcaaaaactattcctaaaaatgtgaagattattgacatagtcaagcacctacattttgctgaaagctacagctattttagctcctaaaacagcgttattttctaccaacttaatatttgtttctaagcttttgccatctgttttttcaacgattgttttaagaaggaaaggtgtagagtcttttccactaattccattggcaatagaatctttaacagcttcttcaattatagtgtcaatataatctttagaaagttcatgttctttaggaacaggatttgcaatgaccattccaccatgtaaatttaactccattttggtcttgaaaatttcagctatttctgtaggttcctcaactgaactatttagttttaaaccgctttctctagtgaaaaaagcaggtagttcagttgtttgatatccaattaccggaacacctttagtttctaagtattcaagcgttttaggcaaatctaaaatagattttgctcctgcgcatataactgtaacatttgtatgcgctagttcttctaaatctgctgaaatatccatactagtttctacgcccttatgaacaccaccaattccaccagtgacaaaaaatggtatcccagctaattctgaacaaatcatagtagaagcaacagttgtagccccaatttttttagtagcaactatttctgctaagtcgcgacgagatactttagcgacattaggactatttgctagagtctccaagtcattttcgtttaaaccaatttttattttcccatccattatggcaatagtagcaggtgtggcgccattgtctcgtattatttgttcaactttttttgccatttcaatgttttgtgggtagggcataccatgagagattattgtagattctaaagctactatgggactattgttttttttggcttcttcaacttctgtagaaaattcaagaaattttttcatttttaaattcctccaattcaatttctaattgtttttgatctaaattttgtctaacagtgtaattagtttcaacagttttcttcgagtttaacaaagctaagttaataatgtcttcattagtataattttttagccaactatatattactgcgctagtaaatgaatcaccagcaccagttacatcaactacatttttagatgaaattactgagtgaaatgattctgaactattatctttgaaaatgagtggttttagtccatttgtaataatgacgttagacacaccaagattaattaatttctcagcagcaatactcatgtcatcattactatcaattttcatttttaaaaaagtttcagtttcatcgcgattaataattaaccaatcaattgaatgtagtgaattaggcatatggatcattttaggtgaagatactggtacaattactaacttaatattgtttttttctgcgaatgaagtgaggtactcaatagattttttgggtaaatttaaatctattactaaacatttagcttttaataagatagatgactgctttgacagaaattcaggtgtaatttcctcgtaaatattcatatctgcaaaaccatactgcatatcaccttttttatctataatagctgtatatgatcctgtacttgcattttctataggttgaatataatttgtattcataaaaggctcagatagttttttaatcaaactccattcgctatcatttccagctgctgttaaaaatgtaacattttcaccaagtctccctaagttttcagcaatatttcttgctacacctccaatcgattttgttgattttactggattggaagtcatagattgtagatcagtatcacaataaaactttctatcaacattagcagctccaatacagattatggaatcttcctcattaacaatgtatgcttttcctaatatatatttcttttttattaaaccagatattatattagctgtggctggccttgataaaccaatacgttctgctaactcttgttgagtaataaaaggattttttttaatttcgtttaaaataaattgctctttatttttcaaaatagcacctccttttaaagaaacaatagttcacaaacaaaacatttgtttgtttcattcaaagagataataacatatatacatttttgtgtaaacgttttcttgaagggttttattttttattctattaaaagataattatactcactttatttactaaataataagatacagtgtttgggacaaaaataagaggctgggacaaaataaaatgtctcagcctattttatcattttgtcagtagctgactgatttgaaaatgcgcttgaatcaagcttttttcaaacctagtcatccttgctggggtaggacaacgaaataaattttgagaaaatattatttctgtcccactcccaagtggatggttattaaatagttgtttgataatctcattattcagtttgagcgtaacgtaaaattgcttcttatgatgctcatcttttcttatgtcaatacgatcgatgattgttagatatagtgatttcaactgagatttctctaatttgtctatatctttgaatattgcttgtaatacattagcaatcatatctgcatcataatgtggagattccgcttgtttatcttgttctagttgatggatttgattatttatttgattcaattcatcttggtagctaagtattgttggtttcaatacgctatctaagtcaggggagtcttcgatagttttcgttagtgtatgcattttggcttttatttcttcacattgtgactgtttataggcaatatcatgattcaaagaagatacgtctatttgacttctttcatttaccttttcaaccaattgcttcaatacctttttgcttttgataatttccaatatctgatccataacatatttttctagtacatctgctctaacactattggctgaacaaacttttgaacctttgtttctaaaattactacatgagtaatatctgattcttttcttagtgccatcttttaatgtattggtcgtattacttgcggccattgctgcaccacatttcggacattttacaatgccagtcagtaggttagtccctttaccgtgaacttgtggtttcttgcgactctcttggcgtttaaactgtactttatcccgtaaagctttatcaataataggcgcatgcttaccatctgcaatgattggttcttcattgagtccttttcgttttttatcgctccagtgtctatacttcgcaaactgtatctttccaatgtaaaaagggtttgagatgatgtaagtaatggacgaaatgctaaaaggtttcgctttcttagtcacataacctttatgattcaatgcgttcgcaatcttacgataaccatgacctttagcgtatgactcaaaaatatatttaacaatattcgcttcatgttgattgatcatgagctcttttttactgtcaggtactttatcatagcctaaaggtaaattaccttggtaataaccttcaatcgctcgttgtctttgaccgttataaacgttttctataatcgtatttctttcaaattctgcgaagctggctaaaatttggagcatcaatttacctgttgagctggcaatttctattttttcagttagactaaaaaattcgacattgattttatacaatttttccacaatatttaataagtctgaggtatttctagctaaacgattggttttgtagaccataatacagtctaacttaccgtcatttgcatcttttaacatacgttgtaattctggacgttccattgttttacccgatataccacgatcggtatattcatcaacgacctcataaccttgaaattgacaatactctgtaagttggtttaattgaccttgaatactgtaaccatttttttgagtttcagtcgatacacgggcatataatccaatatgtttctttttaagttgtttcatattacttccatcctttcagatattattaaatgtgattgttcaacgatattgagtggactatttttaaagtagataccttgtaattgtttagtttgagttattgtaatgtcattaatcaaaggtgctatggtttctaatgtcaatttatctttgattatatgacggattgtttcggtaatttgtttatgtgaataattagagtaacgttcttctctttcaaagccagcagataaacgtttaaacgtttcgatatcaatttgattttgtgccagtttttcgatgagttgttcttgtgttaaatgtgattgtctgtgtttcatttgttggtgttttagagcttttagtattgtcttatttaatttgtcatgaaatgacggattatcacaatatgctttacaagtgttgaggacctctgtttcaatcatttgcgcattgatacctttaaatggacacgtatgataggcttcattcatattcttaggacaaacatagtaacgtagggagtgtttctctttttttatcgttaagtttgttaatgttgattgacagtaaggacatttgattcgtcgctttagcttatttctagaattggatcgattgtgttgcttatgaatacgacgctcttgtgcttcttcaaacatatcaacatcaataataggcggaacgatatcattaaatgtgccatatttattaatgacacgaccgcaatagttaggattcaagagaatatttctaacttgatagggcttacgaggaataagcttaggatggttatctaaatgttgggaaatctttttgtagcctagaccgtgtaagtaccagcgataaactgctttgactgtataggcttcttcttcatgtacaacaaaatgaccttgtctataacgatacccaaaaggtgcatgagttgtgattagcttaccttgtttggctttttctcttgtcccatttcgtgtctgttcactgatattattagactccatttcagctagactcatgagtatgtttaagcgaaagcaatcaaacttttaagacaaatcaaaatatccatcgttaacactgatgattgtgacgtgatgctttttacaaatttcaaagaattgtatggcatttttcaaattacgatggagccgatttaagcgatagcaacataatactttacattttccagatgtaatcatttctaccattttttgataacccgaatgttttgtatgtcgacctgttttcttatcatcataaaatgttacattggaccatccatattgcttagcagtgtctataatgagggatttctgagtcgctaagctttgttgtttgagtgtactttgacgtacataagcaataacttcttccatgttatacacctccaaaaagataatatatatttgtgagtaaattcaaataaaggtccaacgtgcttctaacacgttggaccgcaatgattaataatcatgattttatttttcaataaagtaattagttagtgatgtaataagtttatatttcaaatatgaattatttaataaatattgtaaaatttcattaagttatttatgataaatataaattaaaacgttatttttattttatagtgaaaggattaataataatgaaacacatgcatttatctgttttagcttatagtacaggtctacatcctgcctcttggagactaccacattcatatgttgaagaagttggagatattgattttcaaattaagttagcgaaattagccgaaaaaggtaaactggatgcattcttcttaggtgatggtcaatatatttctggagaagaaacaggacatatttcttattattttgaaccactaacggcgcttgctgccatttcacgtgaaacacattcaattggtttgataggtaccatgtcttcttctttttatgaaccttatcttgcagcacgtatgctttcaagtttacatcaaatatctcatgggcgtattggggcaaatattgtaacatctcaatttgatttagaagcacaaaactactcgatgcaagctttaccacatcttgaaaaacgttatgaacgagcagatgagtttattaatgtaatgaaaaaattatgggaatcatttactgtagaggctatcgttaatcacaaaaactcaggaattggcttaaatcatcagtatattcatccacttcattatcaaggaaagtattttcaagttgccggagctattaacattccaacacccaaatatggtcgaccacgtttatttcaagcaggaacttccattccaggtcgtgatttagcagtacgacacgtggatgctattttttcaattgcatggaatttacaagatggccaacagttcagacaagacattcatcaacgtgccatggaagcaaatcgtcaaccccctcttgtattaccaggtctcactgtttatgttgatgagaatgaagaggatgcttataaacttaagcaacaattagatgatatgattccacttgaaaaacgcaagaaacaattatctaaagctattggtctagatataagtgaatggaaactagatgaagttataccgtccttaccagattatgaaacattatcgaaaaaggtcgtaaaatcagtatatgaagccatacaacgtgccattaagactgagcatcttacattaagagatttattagatcgttttggtacttgggtagggcacaagacaatagtaggaactcccgaacaagtggcggatgaaatgatcgaatggtttaaaaaagaagcgtgcgatggttttatgttgatggccccgacgtatccagaatcatttgaaaaatttattcatttagtgataccaattcttcaagaacgtggagtgtttagaagagattatgagagtcatctgttaaaaaatcatttgggtataaaaaactaaaaataaaccgcatcattaaccgatacgcagaagcttatcacaaataaaactaaaaaattggtaagtagatgaagagtgtaaatcagagtaattaataataatgtatcaaatttaaacaaaggggtctttaagtatgaatttaagaggtcatgaaaataggcttaaatttcttgagaaatatgatgtgacacctatatcacatttaaaattattagaagatcaaaagaaagacggtgaaggtggcatactgacagatagctattactgtttttcatacagcttaaaaggtaattctaaaaaagttttaggtacgtttaattgtggttatcatattgctgaagacttactaaaattatcaaatcaagacaaattacctttgtttaacccgtttaaagtaattaatgaaggtaatcaattgcaggaagtagcgaataaaggtaatttagatattaataggcaaagaaaacagtataatgaagtagctttacagctttcaaatgctataaatttaatcatattttgttatgagggtaatattaaagaaccactttcaacaataaaacacgaaaccgataaatattattatagtaaaccatatgatcgtaaaattaaagcagtaaatactattatcggtaatttgtttgataagaaattagttgagaaaatatctgaaattaatggaaatcaggaaattagaaaatttgatttttcattactcactgatgtaattaaaaaacacgagatacaaaataattttgaataataagtggatgtaagaagatattaaatattgaagctagtattaaggatattcaaaatattataaattattttactgaatgtggcgtgaataataagtattatgagagtgagaaaagaagtagtctaggaaagttggtaagtgttattggacacgaagaaaatgttagaaatccaaaataacctgaattagattttgaagatttcatatctgaatgtataagtgaaaaacaaaaaagaattagacataaactaggaggcagagtatgatgtcatcgaatgagatagtaaaaaaattatattcaaaggaagatattcgcatagaattagagctcactccacataagtttaaaaaaagaatggaaaccattactaagctttttaaaattgatatgaaaatttttcacaattacaaaggccaagataaaaataatcaatacacatttaatggcgtcgcaaaagaattaataaaggtgctactaaaaagtattgactattacccagtggatataaattccaaagcttttaaacaaaacggaaaatctaaaaaagagatgattgaaaatataaaagcatctagttacatggaatatacttatcagttaatgaaatctatcaatgaaattaaatacaaaagattaattgcagacatacatacgaaagacgtatatcaaaatactaaagcatggttaagtattggtgaatcaattaataaaaaggaacaagaattataccaatatatgacacctttgcccatacataaaagaattgagctacaaaatgaagtattaaaatctatagatgaaacgatttttcaatttatggcaaaagaacgtagaaacacccaaataaaagaaaataatgaattagaagaatacacaaatgcaataaaagaaggtaagtatcccaaaaaggattacgaattaaaccacctattatacgagaaaaatgaaatgccattagatagcttaattaaagatgtatgggactatgatgaaacagagtatatggagcttgattggttaattgcagatatgctaaaacgttcacaaagagctgatagtaattttatcgaaagtttagataagaaaaacaaattgagaaaaaatattcataaagaatctattaaaagtatatctaagttgattgatcatgaattggttaaaaataatagaaagtgggacgtagcagaattttataagaatcaacaattttggaacaatagtacattaagacgtagctctcaaaattttgggattttatattacaaaaaaaataggttacatacaatgaaccaaagtaatattattaaaaaaataaaaattatcgaggctaatatagagagtgcaaataaacagccgagctatttagatttctttttacaagctaagtttgacttagagaggttagaaagtgaattaatgaaatatagcattaatccgaaatattttaataagataaatagtgattacgtaagatatgctattgaagatgtacataatgcaattattaaaattgacagatatataagtaacgataaagtgaagttaaactattcaaatgcccaaatggtagtgagaaacgaaataacagaacaaggaagctactttgtaaaccaggcattgaatacactgtcaaaggtagaagagtctggctacagctttgataatttcatggtaggacctttcgtagaagactttaaaaaagcaattaaaaatcgtagatttggttctaaaacagattaagattgttttttagagttaaacataagaataaatttaaataaaaaaacaaacccaacaaaccttgttatatcaacgtttgttgggtttatttttttggtgattttttaataactcaattacaccttagtataatattgctaaattatacattgtcgaggccaagacaaataaaaaattaaagcaaaagttagcgcgcaactttctgccataaaggagcagatttatatggagacaagagacaaactgatgtcattgactcaaagtgacaaaacacaacaatggttaatgaacaaatcatctaaccaaactgatgttcaacaattgcagcaacaattcagtcagcagcttgaccaacaatataatgcacttttagctgatgaacaagctaaattagatcaatatgtggaagtccatcatgaattggaagcattaaaggaagaaattgaagcagaacctattacacttaatattgataaattacccgatatcaaagcgataatgcttgaaaaggctaagaacaatgaacattctgataaaatcgaacagttatttgatagattagatcagtcattaaatggtacgaatcgattatatacacaattatcgttgattggtacacgaacacatcgaatcacaactaaaaattttaatattcagggcttacctaaagcagtccaatgcacgattttaccttcaaaatataagaaggtatatactgtcgattttaaatcatttgaaccttcggttgttgcgtacatgactcaagattcaaaactgattgactttttaaatcagaaagacggattgtatgacgcattgctaagtgaattaggcttatcatatgagctacgagtatttgttaaacgtgcatttattggttcgtttctatttggtggcaacttcgatagcgctaaattcaagttgaaacaatatgtaagtgaagtgcaatggttggatgcggtcagccaatttacaaaagtcattgaacttaagaaacaaatcgaagagcataaaaccattcctatgccttatggcattgaacatgatatgagcgcatttcaaggtagcagtattatagcattttatgtacaaactgtagcgagttatgttttcaagcatattctgttggaagtgtacaaagcacaatgcgaacaaaaaacgtttaaaattattgtacctatacatgatgcgattatgattgaatgtgatgatgaagaaacggcgcaaaatgtatcgcagctaatgaaaagtaaggcaaatgaattgtttaatggtgagtttgcacacgtgacagtggaagcattagggggtgtaaacaatgaataatgatagaggaaaaagtttacaaattccaaaaagcatagccctaactgaaggatatatatatgttgcttcattatattctgtaacccaaacagatttcaatggggatgttaaacatcagtttacgtatgaaatagaggtagatcagaaagttatttatgtaaatcgtagtatttcgaaagatgctaccgataagcagttgtcaatcaatgattggcttaaacatcacagtaattatagctccactcataagaattatgccccctacattgatagaaagcatttaatccatgtaggttgctttaacggtaattattatgtacaagatgtagcatcattaaatgaagatggaggattattataatgaaacatatattcgatatgttaacaaaaataataagtgtggctaaggaggcagtcgaccgtcaaggtctgattgctatcctaaccatgagtattggcaatgatgatgaaatagaagaaacggtacaaggtgaaacagtgtataacgaacttatcgatcagttacgacttaatatcccaaaagatacggattatcgacctaacatctatagctatttcggtattaagaagaaaccaagtgacacaatattaatagacatgatgataaaagtttttcatatcaaacgcttcaattcggaactgtatatattcaaaattaacggttggcaaaagctaagtgaagacgagttaaaaggatttgtatcaaaaatgatacaagtactgttaatcggttatacgcctacgcaaagtgcactgaataatgtggttgaaggtctgcaaaaatcaacagatgtagaagaacttgtcgagaacgagcactatattggttgtggtgaaaatatgttcgatcttaatacattcaaagtcgttaaaaattcaatcgacatttttccaaaaacgcgattaaatttagcgttagataaaaatgatgagattactgaccagatacccaaacatttcaatcaatatatgttagaacttgcaaattatgacgatgatttacaatactttctttttcaacatacagcagtgttattgacggctgatactaaataccgtcgaggtctcatattatatggtggagctaagaatgggaaatctgtatatattgaactagttaaatcatttttctatagcaaagatattgtgtctaagccacttaatgagcttgaaggtcgctttgacaaagaaagtttaattgacaaaagtctaatggcaagtcatgaaatagggcaatctaggattcaagaacagattgtaaatgacttcaaaaagttattatctgtagaatcaatgcatgttgatcgtaaaggaaaaactcaagtggaagtcactttggatttgaaacttatttttagtacaaatgcggtacttaattttcctcctgaacatgcgaaagctttggagcgtcgaattaatattattccatgtgagtattatgttgaaaaagcggacacttcattgattgataagctccagagtgagaagaaagaaatctttctttacttgatgtatgtgtatcaacagattgtaaaagcagatatcgagtaccttgaaaatagtcgtgtcactgaaattactcacgattggttaaattttggatatgaatttgtttctagcaggtccgcaagtattgcaaatcagaaagagtgtattaatttactcagaaaacttatagaaatcaaaccaggatcacgaatcaaagtatccgagttaaataaagttattaatgaagaaataaaggtgagttctcaggttattaaacagttaattcaagaaaactttgatactcaaaccaaactatacaatggctacgattattggattgatttaggttggaaagaagccgataaaaaagagattcatgatatttcgaaaaaagataatattatttcattagaaaaaaatgaaaatataacagacgatgaggcattagatgaagagaatttggactttgattgggaggactttgacgatgaataatgaacaaattgaagcatttgtagaagtacttgtgcctatcatagaagaacgtatcaataaaggtaagtaatctaattacgtactacaggcagttgcctgtagtactcatatgattaagtgggaaaagtgataaaaatgaaacgaaattataaatatatattatccatatgatgttacaagaccgatggtctgtagcaataatctaataaaaggagcggtatgatatgaagggtaaaattgcactttattcacgcgttagtacgtcagagcagtcggagcatgggtactcaatccatgagcaagaacaagtactcatcaaagaggttgtgaaaaactatccaggttatgactatgaaacttatatcgattctggtatatcaggtaaaaatattgaaggtcgaccagcaatgaaacgtctattacaagatgttaaggataataaaatcgaaatggtgttaagttggaaattgaatcgtatctcacgatcaatgagagacgtgtttaatattattcatgaattcaaagaacatggcgtagggtataaatcgatttctgagaatattgatacatccaatgcttctggtgaagttttagttacaatgtttgggttaataggatctatagaacgccagactttgatttccaatgtgaaactttctatgaatgctaaggcacggagcggagaggcaatcaccggtcgtgttttaggctacaaattatcacttaatccattgacacagaaaaatgatttagttattgatgaaaatgaagctaatattgtacgtgaaattttcgatttatatttgaatcataataaaggacttaaagcaatcacgacaattctaaatcaaaaaggatatcgcaccattaatcaaaaaccattttcagtgttcggcgtgaaatatattttgaataatccagtctataaaggttttgttagatttaataaccatcaaaactgggcagttcagcgaagaggtggtaaaagtgatgaaaatgatgtgatattggtcaaaggtaagcatgaagccattataagtgaagatgtatttgatcaagttcatgagaaactagcttctaaaagttttaaaccgggtcgacctattggtggagatttctacttacgtggtcttattaaatgcccagaatgcggaaataatatggtatgtcgacggacttattataaaacgaaaaagtcaaaagaacggacaatcaaacgctattacatttgttcattatttaaccgttctgggagttctgcttgtcatagtaattccatcaatgctgaagtcgtcgagcgtgtaattaatgttcatttgaatcgtattctgtctcaaccagatattatcaagcagattgcgtcaaatgtgatcgaagaactgaaacaaaagcatagtaaccaaacagaaattaaatatgacattgatagtttagaaaaacaaaaagctaagcttaaaacacaacaagaacgattattagatttatatttggatgaggaaatagatagcgaaatattgaaagataaacaaagtcaaatgaatcaacagttagaagtattagatcaacaaattaaagaagcgcaacaagcaaatcaatcacaggatgaaatacccaattttgataaattaaaaggacgactcattttgatgataacacgattcagcgtgtacttaagagaggctacacccgaatctaaaaatcaacttatgaaaatgttaattgattcaattgaaattacgacagataaacaagtaaaacttgtaaggtataaaattgacgaaagtcttatcccgcaatccattaaaaaggattgtgggaatttttttatgcctaaatttaactttgtgataaatgtcacaaataaaaataggattgaaaatttatcacttttaccacttttttagagtgacaaaagtggaggagttttgaaatattttataaatatatattttatttatggagtacacattattaattaaggaggtcattatagtgacgctaagcaaacaacttaaaacgtatattactgaacgatttaaattaaattatcaagaaacttggagttgtgaaaccgtagacgcggtggctgaagacgtattacctgaaaaatatattaaaaatagtccactcgaacataaaatattgaacacatttacttattataacgatgaattacatgaaatcagtatttatcctttcttatactatttagataaggaattaatagcaataggttatttagataattttgatttagactttatatttttaaatgacactcatcaaattattattgatgaacgctacttgttacaaaaagggggcgagtaattatgaactggattaaggttgctcaactatctgttacagtcattaacgaagtgattgagatcatgaaagaaaagcagaatggaggaaaatagtatgaacatcaatcgatacatcacaagaggcattagtgaacaactatctctagaccttcaaatcttactttggcacatggtagaagaaaaagataaccagcctcataccgattacctacacattttcaaactacaagatgatgataatatgttgtcaattacacatgaacaagaacagcccgtatacaagttagaatatcactatacaaactatgaaaaaaatcaaaatgcattacctaagaaagtctacgtcattcgtgaagatgatgtagacgttttttattatgtgatgcttttaccagaagaatactaaaaggagtgacgttgatgaatacaatcaaaagtacgatacacacagaagctatatttagcgatgatgaacaacaccgctacttactcaaaaagacgtgggatgaaaagaaacctgtttgtacagtgataacgatgtatcctcatttagatggcgtattatcactcgatcttactactgttcttatcctcaaccaattagcgaattctgaacaatatggcgctgtatatctagtgaatctattctctaatattaaaacaccagagaatcttaaacatattaaagaaccttatgataaacacacagacatccatttgatgaaagcaattagtgagagtgatacagtgattctagcttatggtgcttatgcgaagcgacccgttgtcgtcgaacgtgttgagcaagtaatggaaatgttaaaatctcataaaaagaaagtcaaaaaactcataaacccagcaacgaatgacattatgcatccgcttaatcctaaagcacgtcaaaaatggacattgaaataaaggaggattatatatgaaccataacactacacaatcagattggcgaatagttgctagttgcttagcatcacaaaattatatatctatcgtaaaaggattagtacatcattttacagcgattgcagatgaggaaacacttgataaaatctatgaagattttatgaatgatgactctataaccacggtacttaataatgatttacagacaattattaaccattatctgtcaaaatgaaaattatattctaataaaactagagcatccttcacttagtggtgagggatgctcttatctttatttttttgattaatattttactcaggaaattttacattaaatttaaaagtattatacaattaaattattagtttctagtgaagaaatacgtattaaatttattattaactgtagcacattatcaagcaattgtactgttaaaagggattggtcattcaatgagacaatatgtttatcaaaatgatattaatttaataaactctttatatgagagtgatttttggaagataataaaagaagacgcagcatattatcataaaaataataaattcaagaaagataatgctatacgaatacttgaatctctaattaaatcaatatatgtagatcctgatggttttgataaagctcttgcagctgaaatgcaagatttctataacaaaatgcaaaaatcacaatacatcaaagagtcttattatcttagtattaatcaccagaaatgtagtctagatgctctcatcggatggaaaccacttttccgatttagaaatggtgataaaaaatggttagatgacttagaacttattagagggaatagaatgggccatttagcttttccagtacaaaaaaattctcttaatcaactaagaggaattttattaaaagatagaattgattatactctatttgatattaaattattttatgaaaatgcagctcatttaaaattacagaaagcttatgaacaagaaccaacacgaaaatggctaaaatcatttggtacctttaatcaatttatagagcgtatgcaattgaactacttcgtctataaagatccaatcacattaaaatatgatgttattgacttatcattgccatataataatgataagtcacattgcttaaaagaaattccaaaaaaaattaaggtcgaagaaacttatattacaaatatacttaattatattaaaaaatatggcgaaaaattatctactatccatgtggacttaatgattgattatcatgtataaataaaagaacaacccttcaccgtaaagtgaagggtgctctttagcttctttcattatttacaaatttcatctctttttttgatacaattctaacttaattaaatataatgctactctataaatctcctacatatttatagctcatatcctctaaaataaccagtgagtatctatacatatattttatggtaacgtaggctttttctagtttacattttattgattactcgctataagttctgtttgctcgacaacttgttcgacagtcatcttttgtaaatcaggaggataaccatattttttaagcaatcgtctaaaagttaagcgcatttttacttttgcactatcgcgtttagataaattgacgcccatattttttcactgttttagttagctcatgagcaattgcacgtagttctttatcaccattgcctctttagttatttcatgtgatgaagctaatgcataataaaatacaaggtccttaattactattgagatgttagaaaatattaaagaaagcaatttttactaaattttaaggacattacgtttttataattaaattaaagttagcttttataagaaagatattcatacttaataaaaaaaaactattaaattttgtttgactaaagttggatagtacattatagtataattacaatactaatgtgtattgtacttatacctaaaattacagaatctactaaaacaaggcaaaatgccgtgtttatctcgtcaacttgttggcgagatttttttatatcaataatataaatttcatgtatctgggagtggtcatatgaaaaggaattatatcttaggattagatatcggaattacatcagtgggttatggaattattgattatgaaactagagatgtcatagatgcgggcgtacgtttatttaaagaggctaatgttgaaaataatgaaggacgacgatcaaaaagaggtgccagaaggcttaagaggcgtcgtagacatagaatacaaagagtaaagaaacttttatttgattacaatttgttgacagatcatagtgagctaagtggaatcaatccttacgaggcgcgcgtaaagggattaagtcaaaaattaagtgaagaggaattttctgcggcattgctacatttagcaaagcgtagaggtgtacataatgttaatgaagtggaagaagatacaggtaatgaattatccactaaagaacaaatttcaagaaatagtaaagcgttagaagagaagtatgttgcagaattacagttggaacgtttgaaaaaagacggtgaagtgagaggttcgattaaccgtttcaaaacatctgactatgtaaaagaagcaaagcagttattaaaagtacaaaaagcatatcatcaacttgatcaatcatttatagacacttatattgatttattggaaacaagaagaacatattatgagggaccaggtgaaggtagcccatttggatggaaagatattaaagaatggtatgaaatgttaatgggacattgtacgtatttcccagaagaattacgtagtgtgaaatatgcctataatgctgatttatataatgcgctgaatgatttgaacaacttggttattacacgagatgagaatgagaagctagagtattatgaaaaattccaaattatcgagaatgtctttaaacaaaagaaaaagccgacgcttaaacaaattgcgaaggaaatcttggtgaatgaagaagacatcaaaggctatcgtgtcacaagtacaggtaaaccagaatttacaaacttgaaagtttatcacgatatcaaagatattacagcaagaaaagaaattatcgagaatgcagagctactcgatcaaatagctaaaatattaactatttaccagtcatcagaagatatacaagaagaattaacaaacctaaattcagaattgacacaagaagagattgaacaaatttcaaacttgaaaggttatacaggaactcataacctttcactaaaggcaataaatttaatattagacgaattgtggcatacgaacgataatcaaatagctattttcaatcgtttgaaacttgtacctaaaaaggtagatttaagccaacaaaaagaaattcctactactttagttgatgattttatactgtctccagtagtgaaacgttcatttatacaatctattaaagttattaacgctattattaaaaaatacggtttgccaaatgatattattattgaacttgcgagagaaaagaattctaaagatgcacaaaaaatgattaatgaaatgcagaagagaaatcgtcaaacgaatgaacgtattgaggaaattataagaacgacaggtaaagaaaatgctaaatatttaattgaaaaaattaagctgcacgatatgcaagaagggaaatgtttatactcgttagaagcaatccctctagaagatttacttaataatccattcaattacgaagtagaccatatcattccacgttctgtttctttcgataactctttcaataataaagtgttggtgaaacaagaagaaaatagtaaaaaaggtaatagaacgccatttcaatatttaagttcttcagattctaaaataagttatgagacattcaaaaagcatattttaaatcttgctaaaggcaaaggtagaatctctaagacgaaaaaagaatatttgttagaagaacgagatatcaatcgcttcagtgtccaaaaagattttattaaccgtaacttagtagatacacgctatgcgacaagagggttaatgaacttattaagatcttattttagagtgaataacttagatgtcaaagtgaaatcgattaatggcggattcacaagtttcttaagaaggaaatggaagttcaaaaaagaaagaaataagggctacaaacaccatgctgaagatgcactgattattgcgaacgctgattttattttcaaagaatggaaaaaactagataaagctaaaaaagtgatggaaaatcaaatgtttgaagaaaagcaagctgaaagtatgcctgaaattgagactgagcaagagtataaagaaatttttataacgcctcatcaaattaaacatattaaggattttaaagattataaatattcacatagagttgataaaaagccgaatagagagttaataaatgatacattatattctacgagaaaagatgacaagggtaatacattaatcgttaataacttaaatggtttatacgataaagataatgataaattgaaaaaattaattaataaatcacctgaaaaattattgatgtatcatcatgatccacaaacatatcaaaaattaaaattgatcatggaacaatatggcgatgagaaaaatccgctttataaatattatgaagaaacaggcaattacttaacaaaatatagtaaaaaagataacggaccagtcatcaaaaaaattaaatattatggtaacaagctaaatgcgcatttagatattacggatgattatccaaatagcagaaataaagtagtaaaactttcattaaaaccatatcgctttgatgtttatttagataatggggtatataaatttgtgacagttaaaaatttagatgttatcaaaaaagaaaactactatgaagttaattcaaagtgttatgaagaagcaaaaaaactgaagaaaattagtaatcaagcagaatttatcgcaagtttttacaataatgacttgattaagattaacggagaattatatagagtcataggtgtaaataatgatctacttaacagaattgaagtaaatatgatagacatcacatatagagaatatttagagaacatgaatgataaaagaccacctagaataattaaaacaatagcaagcaaaacacaatctattaaaaagtattctacagatattctaggcaatctttatgaagtgaagagtaaaaagcatcctcaaatcataaagaaaggatgattggatattggcatggagaattgtatatctttcagaagtagataagcttgcattaaatttaaataacttaaaagtcgcaaaaggggatttggaggtaaaaatcccccttagcgatattttcgcaattgtgattgaagatttaacaactactataacctctaggcttatgatagagctatctaaatacaatattttagtgattttttgtaatcaaaagcatttaccagagtgcatgattcaaccgattaatggtcattttaatcaatatggccaaatgaaggaacaactacaatggtcggaagaaagaaaagctgaattatggaaacatattctgtttcaaaaaatacaaaatcaaattcagtgtatgaaacattttggagtggatgaagaaagaataattaaaatgaaaaaattacaatcaatggttacatctaaagatgaaatgaatatagagggccaagcggctaagtattattttaatacatttttcaaggacttcagacgcgatgatgattttttagtagaaaatatggtactggattttgggtatactattttaaattcagcaatcgcaaggaccattgtagctaaagggttaattccagcattgggaatacatcatattggcgcaagaaaccactttaatttagcatcagatatcattgaagtatttaggccattggtagatttatatcttttgaaacatcctccgaaagtggaatatatgactagagagtatagattagagctgattaacttgctgcatgctagagtacaaattgatggaaagcagcatacagttattagagcgattgaaattatggttcaatcaataattgagtattttagaacggggagatataaaacgctcaaattaccaaatattaagcaatattcattttataaatcatgagttataagtttatgagagtaatgattatgtttgatctcccaactgacacaaaagaagaacgacggttatatagtaagtttagaaagggactcatttcggaaggctttttgatgatgcagtattctatttacattaaatgttgtattaataaagatgcggcaaatagtagtgtaaattatgtgaaacgtattttaccaccaaacggacatgttagagctttaacaattaccgaaaagcaatataaaaaaatgaaaatattattaggagatgaagataaaaatatcgaaatattaggagataatcgtacaattttattttaggagaaaacctatgtatgaatcaattttagaaatcaatattgatatggtacccaaagttattttaaatactagtgtatatacatctatatataatgaagattcaacacatgaagaatatattttagatatgcttaagaattattttcaatctagaaattcaaataaggatattgttacgattacagatatttcagatcatgaaagagtatctcataatcggtttagaggatttctcttagatcattctactattgaaaatgaacaccaattatcatcatcgagtattttgactaagaagattgttagagaaatgcaaagtgatttggaaatagatggttatattaattctatcaatgtactgttggatgacttacgagataatttaaagggcacactgccactttctattaagtctttcgatttaaaacaattcataaagctactctcatttaaatatgattattcggaagattatgccagactaattactcggttagaacaagtcgtcccattagtagtggatgaaatgaattatcaagtaaaagaaaaagcatttgtaatctatttatatccagaagctggcctaagcattaaagaacaaataagatttagaaaaatactaaataacttacctgttccggtcattgttctaaccgaatcaccacgttttttatctgaaagtattaaaggactaaattattttattaataatgttcaaatgatcacagaatctttttttgaagatagctattggaatgcaccaattaatgtagaaaaagaacagattgaagagaggtttgaatatttatttgtaaaatattgttcagttttagaaataaaaccgattatttctaactatttacttgcggatatcattgtttttaatgatattgatctttatatccttgtttcatttttgaaacactgtaatttagagtataaattagatatcgataaaacaaaaatttcattagcattatcgtcatatctattttcttaattattttgaggatttataatgatgctagaggttttagtactctgtaattttaggtatgaggtagaccaggtttgtacccactgacaccaacaagcggttttagtactctgtaattttaggtatgaggtagaccgtaaagactttaacgaatttatggataaagttttagtactctgtaattttaggtatgaggtagacaggaacaacctgatttaaatatgtggttgggttttagtactctgtaattttaggtatgaggtagactgtagcttcttcaagttctttaaatagttcgttttagtactctgtaattttaggtatgaggtagacaaagtggcgatgttattaatatcaaaggttgttttagtactctgtaattttaggtatgaggtagactaatgtttgcggtagaaggtttacctgtacgttttagtactctgtaattttaggtatgaggtagacaagttggtgaaattttatataacgcaaacagttttagtactctgtaattttaggtatgaggtagactaacgcatgtgtaatggttctaccctgccagttttagtactctgtaattttaggtatgaggtagacccactgcaacaagtcgtcgtgagcgtgtgcgttttagtactctgtaattttaggtatgaggtagacaaatataacgtggtttattacgtcagacgggttttagtactctgtaattttaggtatgaggtagacaaataccaaattttgaattgaacccaaatcgttttagtactctgtaattttaggtatgaggtatatcttttttaggtcggctttttattttgaatagttttagtactctgtaattttagatatgaggtatatagcaaaatcactgatagggagaggcgtatcataagtgatgagtttgtttattataagatatacgaaaaatattaatttaaagatatcagagaaacatagagtatttatataactgtttagaagtataaaataatcattttttgtatcatacagttggttctataatgaatcactaagaatgattgtattcaataaattaataaaaagcatatacatggtattagcaaatagaaattaactaggttttattggtttatagcctttaaataaatatatttaatttaaattcgcgattaggtagtagtaattaatgtttgagattgaaaatagatttaaatatagcaattatatattaacctattaaagtgttaggctataatgattagaatattctaggagatataaataaaatgaggaaattatacaatttaaaagaatttttaaatatttattcaactgaagatataggtttaattaatacatatatcgaatctgataatagaccacttaaagaaaatgaagtagaggatttaaaatcattaataaatctcttgaagctaaattataaaagttgtgaaggtttttttcttagttatgaagttcctcatatcggtcacgaaatagacttattgaaagttacggataatgctattttaaatatcgaattaaaaagtagatctgagcttgcaaagataaataaacaacaaaagtataattatttttatcttaatacacttaacaaaaatgtagacattataacctataatagacatgaagaaaagttttataaatattgtcaagaaagtgagaaatcacttgaaataaatatagataaagtaagggataaaatttttgaatatggaaataaagagtttatttcagatattgattatttatttaaaccttctaatttccttatttcaccttttaatgatactgacaaatttcttgaagacaaatattatttaacggcccagcaagaaaaaataaaaaaagacattataaatcataatgggactattgctattattgaaggaagaccaggcacaggtaaatcacttttattatatgatattgctaaaaaactaaaaaaagagtttaatatattaataatacattgtgcattgttaaatgaaggacacgaattaatgattaataaaaattggaatataaaaagtgctcataaaaattgggtatacgatgaagagaattatgaaggtaaaaattatatttttattgatgaatcacataggttttaccctaaacaatttgagtatgtaatagaaactgcacttaaaaaagatattaagataataacaactatagacccattacagtatctaagagataatgaaaatgattttgaaaacttacagagattaaaatctcattctaacatctattataaaaaaattgataataaaattagatctaatccagaaatatcatcatttgttaaaagtattattaatttaagaaatatacctgaatataaatttaagaatatttcaatagaatatttgtcaaaagaagatgattggaaatcatatttgctaaatttacgtgatagaggatggacatatttaccttatacgaaaagtagagataatattagttatcataaatattgttcggctaatactcatttaaatactcatagaattattgggcaagaatttaataaagttattgttattttagatgaaggatttaaatatgttgatggatatttaggatattacggagattattattataatcctagacaaatgttgttccaaaatttaactagagctagagaaaaaataaaaattataatcattaataatacagatttatataaaaagattaatcaagtgttaactaagtcttctaataaaaatgagttatcacttaaattttttattcctgaacttaataatgataaattaaaatcattttatagtgatattttaggttttaagttaattagtaatcaaaaacaaccgcctggaaaaagaaagataagttttcaaataggtgaaacaaatttagggttttatgaaaaaggagatatttctaaaaacaataaatgcgaaataaatatagttgtaagtaatttgaaagatttaaagaaaagaatatcaaatgaaaatatggtattgattagtgaagaagaaggtaaaaaaagtaaatttgttactttaaatgatccattaaacaactatttaaagttaatagagtatatataactagtattttgaattatttaaagatttattgaagttttgatattaatttgtcgaaaaacgaaccaaattattaaatgctacacaaaagaatatcaagtataagttattaatcataaatcagattgggtactcacctattggaagtgaagatgccaaactattattccaattaatagatttaaggtatgagaagaaaagtacaatagttaccacaaatatcaaattcaacttatgtaacgaaatatttgatgattccaaaatcgcaaatgcgattttggataggatattgcatcattcaagcgtagttaaaatcacaggtaaatcatatagattaaaagatcattcacctaagaaggaaattacttagcaaacaattttgtacattcttatacaatcatttatgtacatttttatattgacatttacaagtaagcaagtgaacttatctgctccagctgtaagagaaagggtaaataaacttgaagagcaaggtattatacaaggttatacaattaacatagattataaacaattaggttacgatgtagaaaaattaattgagttaactataaagaataatagatacagccatatgggcagacaaaatgtcagtttatcttttcatcagttgtctaaactacatggaaaaagtttaataagcataggaaagatttttaacagagagaagtgacttattttggaatataaatcttacaacaaaatgagtaataatattttatctatcttgttaagtgaaaaaaatttcgataataaaatggtagtctcaacaggtagttatattttgtctgagttgccatgtattgttgcctataaaaataatgatattgtggggctactaacgtataaagtttatgatgagtacattgaaatcatttctttagatagttttgtagagaacaagggtattggtagtcatttacttaattatgctgaaataattgcctcagatatgagtaaaagaagtatccgtgttattactacaaatgaaaatattaaggcactctatttctatcaaaaaaataaatatagaatcacagacgttatttttgatgctgtaacagaagctaggaaaataaagccgtcgattcctacaattgataaaaatggcattgaaattagagatgaaattgttttgaggaaatgtttgtaatgtataaatacactcagctttaaatcaccctagttcatacctaaaagactttaacacaaacaaaaaaggaggaacattaaattcctcctcaacctttattactcatactacaattctattttaacgtcttcgtccatttgggcttcaaattcatctagaagtgctcttgcttctgcaattgattgtgtgttcatcaattgatggcgaagttcgctagcgcctcttatgccacgcacatagattttaaagaatctacgcaagctcttgaattgtcgtatttcatctttctcatatttgttaaacaatgatagatgcaatctcaacagatctaatagttctttgcttgtgtgttcacgtggttctttttcaaaagcgaatggattgtggaaaatgcctctaccaatcatgacgccatcaatgccatatttttctgccagttcaagtcctgtttttctatcgggaatatcaccgttaattgttaacaatgtatttggtgcaatttcgtcacgtaaatttttaatagcttcgattaattcccaatgtgcatctactttactcatttctttacgtgtacgaagatgaatagataaattggcaatgtcttgttcgaagacgtgcttcaaccaatctttccattcatcgatttcatagtagccaaggcgtgttttaacacttaccggaagcccacctgctttagtcgcttgaataatttcggcagcaacgtcaggtcttaagattaagccggaacccttaccctttttagcaacatttgctacaggacatcccatatttaagtctatgcctttaaagcccattttagctaattgaatactcgtttcacggaactgttctggcttatctccccatatatgagcgaccatcggctgttcatcttcactaaaagttaagcgtccgcgcacactatgtatgccttcagggtggcaaaagctttcagtatttgtaaattcagtgaaaaacacatccggtctagctgcttcacttacaacgtgtcgaaagacgatatctgtaacgtcttccattggcgccaaaataaaaaatggacgtggtaattcactccaaaaattttctttcataatatatttataccctct

SEQ ID NO: 50 - DNA, 23 bp, Bacterial
cctggcctgccccaagtgcaagg

SEQ ID NO: 51 - DNA, 32 bp, Bacterial
gtcgccccccacgcgggggcgtggattgaaac

SEQ ID NO: 52 - DNA, 28 bp, Bacterial
tggagcgggaaacgggatttgaacccgc

SEQ ID NO: 53 - DNA, 29 bp, Bacterial
gtgttccccacgggcgtggggatgaaccg

SEQ ID NO: 54 - DNA, 25 bp, Bacterial
aacctttctgcaaaaaggtttcccc

SEQ ID NO: 55 - DNA, 23 bp, Bacterial
ccgctggatccggctgcagcgcc

SEQ ID NO: 56 - DNA, 28 bp, Bacterial
gttcactgccgcataggcagctcagaaa

SEQ ID NO: 57 - DNA, 32 bp, Bacterial
cacccgactattgaagtcgggcctcattgaag

SEQ ID NO: 58 - DNA, 36 bp, Bacterial
gtcaaaacccataccgatatggatacctcttttgag

SEQ ID NO: 59 - DNA, 36 bp, Bacterial; identical to SEQ ID NO: 58

SEQ ID NO: 60 - DNA, 36 bp, Bacterial; identical to SEQ ID NO: 58

SEQ ID NO: 61 - DNA, 36 bp, Bacterial; identical to SEQ ID NO: 58

SEQ ID NO: 62 - DNA, 36 bp, Bacterial
ctcaaaagaggtatccatatcggtatgggttttgac

SEQ ID NO: 63 - DNA, 28 bp, Bacterial
gttcactgccggataggcagcttagaaa

SEQ ID NO: 64 - DNA, 32 bp, Bacterial
gtcgccccctgcgcgggggcgtggattgaaac

SEQ ID NO: 65 - DNA, 29 bp, Bacterial
ttttctgagctgcctatgcggcagtgaac

SEQ ID NO: 66 - DNA, 46 bp, Bacterial
catcgacgacgaacccgggcaccgcctgatggtccacgccgtcatg

SEQ ID NO: 67 - DNA, 32 bp, Bacterial
gtcgcccctcacgcgggggcgtggatagaaac

SEQ ID NO: 68 - DNA, 32 bp, Bacterial
gtttcaatccacgcccccgcacggggggcgac

SEQ ID NO: 69 - DNA, 28 bp, Bacterial
tttctgagctgcctatgcggcagtgaac

SEQ ID NO: 70 - DNA, 36 bp, Bacterial
gaccgaagacctgtcggaaacgacggggattgagac

SEQ ID NO: 71 - DNA, 29 bp, Bacterial
cggttcatccccgcgagtgcggggaacat

SEQ ID NO: 72 - DNA, 28 bp, Bacterial
tttctgagctgcctgtgcggcagtgaac

SEQ ID NO: 73 - DNA, 29 bp, Bacterial
gttttatctgaacgtagtgggatataaag

SEQ ID NO: 74 - DNA, 29 bp, Bacterial
cggttcatccccgcgggtgcggggaacac

SEQ ID NO: 75 - RNA, 28 nt, Bacterial
guuagcagccgcauaggcugcuuaaaua

SEQ ID NO: 76 - DNA, 33 bp, Bacterial
aatttaaatagggaagataagcaaagggttgac

SEQ ID NO: 77 - DNA, 31 bp, Bacterial
tttaaatagggaagataagcaaagggttgac

SEQ ID NO: 78 - protein, 11 aa, Bacterial
NLNREDKQRVD

SEQ ID NO: 79 - DNA, 32 bp, Bacteriophage
cattgcaactatgcaaaatgatgaagctaaaa

SEQ ID NO: 80 - DNA, 32 bp, Bacteriophage
tgttagagtcggtagtatctggatgatcgata

SEQ ID NO: 81 - DNA, 32 bp, Bacteriophage
ttatgtattgaccccgacacgccccccgactg

SEQ ID NO: 82 - DNA, 32 bp, Bacteriophage
ttacagacgacctaactcttcagtaccatgat

SEQ ID NO: 83 - DNA, 32 bp, Bacteriophage
tacataagctgcaacacggtgttcgtttaagt

SEQ ID NO: 84 - DNA, 32 bp, Bacteriophage
aaaatacgcctttttcccttcatcgtttaaag

SEQ ID NO: 85 - DNA, 32 bp, Bacteriophage
accaacaaatcccataaactgataaccacgtt

SEQ ID NO: 86 - DNA, 32 bp, Bacteriophage
gtcaaccctttgcttatcttccctatttaaat

SEQ ID NO: 87 - DNA, 32 bp, Bacteriophage
tgttaaccaccgcttgaaataatcatgatgca

SEQ ID NO: 88 - DNA, 32 bp, Bacteriophage
tgtgtctatactcaaccaatttaagcgccgca

SEQ ID NO: 89 - DNA, 32 bp, Bacteriophage
ctactctccccaatattagccattcctaattc

SEQ ID NO: 90 - DNA, 32 bp, Bacteriophage
gtcaccttaccgtaagacaggcagtaaaatta

SEQ ID NO: 91 - DNA, 32 bp, Bacteriophage
aaactagtggacgtaatgcagtattcacggtt

SEQ ID NO: 92 - DNA, 32 bp, Bacteriophage
atccacactacaaatagaacactcaaccgtga

SEQ ID NO: 93 - DNA, 32 bp, Bacteriophage; identical to SEQ ID NO: 88

SEQ ID NO: 94 - DNA, 32 bp, Bacteriophage; identical to SEQ ID NO: 89

SEQ ID NO: 95 - DNA, 32 bp, Bacteriophage; identical to SEQ ID NO: 91

SEQ ID NO: 96 - DNA, 32 bp, Bacteriophage
ataatcgttttgagtctcaccagcttttaggc

SEQ ID NO: 97 - DNA, 32 bp, Bacteriophage; identical to SEQ ID NO: 92

SEQ ID NO: 98 - DNA, 32 bp, Bacteriophage
tattgattggtctctaaccttgggatgattaa

SEQ ID NO: 99 - DNA, 32 bp, Bacteriophage
ttcacgggtagcaacagggtaataaaccaata

SEQ ID NO: 100 - DNA, 32 bp, Bacteriophage; identical to SEQ ID NO: 79

SEQ ID NO: 101 - DNA, 32 bp, Bacteriophage; identical to SEQ ID NO: 80

SEQ ID NO: 102 - DNA, 32 bp, Bacteriophage
tagaagagtaataggagctactgcaaacttgt

SEQ ID NO: 103 - DNA, 32 bp, Bacteriophage
taactatgtgtggtttatattttgtgtgcaag

SEQ ID NO: 104 - DNA, 32 bp, Bacteriophage
ttttgaaactattgacagaaggttgggaacct

SEQ ID NO: 105 - DNA, 32 bp, Bacteriophage
ttgaggttgaacctcttccggttcctcttctg

SEQ ID NO: 106 - DNA, 32 bp, Bacteriophage
gtgtattgcttgcagtgggttacacacaagaa

SEQ ID NO: 107 - DNA, 47 bp, Bacterial
gttgtgatttgctttcaaattagtatctttgaaccattggaaacagc

SEQ ID NO: 108 - DNA, 29 bp, Bacterial
atttcaattccataaggtacaattaatac

SEQ ID NO: 109 - DNA, 32 bp, Bacterial
gtttcaatccacacacccgtatagggtgtgac

SEQ ID NO: 110 - DNA, 47 bp, Bacterial
actgtttctgatatgtcaaagataaaattttgaaagcaaatcacaac

SEQ ID NO: 111 - DNA, 23 bp, Bacterial
gaaaaaatacagtttcgctctca

SEQ ID NO: 112 - DNA, 32 bp, Bacterial
gtcgcgtctcacgtaggcgcgtggattgaaac

SEQ ID NO: 113 - DNA, 47 bp, Bacterial
attgtgcttgctactgcaaagatacacattttgaagcaattcacaac

SEQ ID NO: 114 - DNA, 37 bp, Bacterial
ctcaatgagtatcttccattaaaacaaggattaagac

SEQ ID NO: 115 - DNA, 36 bp, Bacterial
gttgtttttaccttgcaaacagcaggcagatacaac

SEQ ID NO: 116 - DNA, 47 bp, Bacterial
gttgtatttgccaatgcaaagatactaattttaaagctaatcacaac

SEQ ID NO: 117 - DNA, 36 bp, Bacterial
gttgtatatcattcctttcctacatcaaaccacaac

SEQ ID NO: 118 - DNA, 487 bp, Synthetiic
gcggataacaattactagagaaagaggagaaatactattcttctcctctttaaataacgaaaacaccctgccataaaatgacagggtgttgatttcggcatgaagccttatctttgtagcttctgcaagatttaagtaactgtgtaaggcgtcccttacacttgcatgtatagttattataccagggggacagtgcaatgtcaagaataaactgtagaatgactagtgacttaaatcttgagagtacaaaaacccgttggaatcgtgattaatagtaactgttgttgtacagttacttaaatcttgagagtacaaaaacggccgagaaaaggagctgattcataggacagttgtacagttacttaaatcttgagagtacaaaaactcaaacttgcccgtagtttatcttatagccgttgtacagttacttaaatcttgagagtacaaaaacatttacctcctttgatttaagtgaacaagtttatcc

SEQ ID NO: 119 - DNA, 221 bp, Streptococcus thermophilus
ttaaatcttgagagtacaaaaacccgttggaatcgtgattaatagtaactgttgttgtacagttacttaaatcttgagagtacaaaaacggccgagaaaaggagctgattcataggacagttgtacagttacttaaatcttgagagtacaaaaactcaaacttgcccgtagtttatcttatagccgttgtacagttacttaaatcttgagagtacaaaaac

SEQ ID NO: 120 - DNA, 112 bp, Streptococcus thermophilus
ttaaataacgaaaacaccctgccataaaatgacagggtgttgatttcggcatgaagccttatctttgtagcttctgcaagatttaagtaactgtgtaaggcgtcccttacac

SEQ ID NO: 121 - DNA, 30 bp, Streptococcus thermophilus
tgtcctatgaatcagctccttttctcggcc

SEQ ID NO: 122 - DNA, 30 bp, Streptococcus thermophilus
ggctataagataaactacgggcaagtttga